European Patent Specification EP 3 436 603 B1, published November 26, 2025. Title: GENETICALLY MODIFIED STRAINS OF MYCOBACTERIUM SMEGMATIS. Applicant: University of the Witwatersrand, Johannesburg. The sequence listing filed with the application follows.

SEQUENCE LISTING (14 sequences)

SEQ ID NO: 1 - DNA, 80 bp, Mycobacterium tuberculosis
gcaccagccagctgagccaattcatggaccagaacaacccgctgtcggggttgacccacaagcgccgactgtcggcgctg

SEQ ID NO: 2 - DNA, 80 bp, Mycobacterium tuberculosis
gcaccagccagctgagcctattcatggaccagaacaacccgctgtcggggttgacccacaagcgccgactgtcggcgctg

SEQ ID NO: 3 - DNA, 80 bp, Mycobacterium tuberculosis
gcaccagccagctgagccaattcatggtccagaacaacccgctgtcggggttgacccacaagcgccgactgtcggcgctg

SEQ ID NO: 4 - DNA, 80 bp, Mycobacterium tuberculosis
gcaccagccagctgagccaattcatggaccagaacaacccgctgtcggggttgacctacaagcgccgactgtcggcgctg

SEQ ID NO: 5 - DNA, 80 bp, Mycobacterium tuberculosis
gcaccagccagctgagccaattcatggaccagaacaacccgctgtcggggttgacccacaagcgccgactgttggcgctg

SEQ ID NO: 6 - DNA, 80 bp, Mycobacterium tuberculosis
gcaccagccagctgagccaattcatggaccagaacaacccgctgtcggggttgacccacaagcgccgactgtcggcgccg

SEQ ID NO: 7 - DNA, 80 bp, Mycobacterium smegmatis
gcaccagccagctgtcgcagttcatggaccagaacaacccgctgtcgggtctgacccacaagcgtcgtctttcggcgctg

SEQ ID NO: 8 - DNA, 962 bp, artificial sequence
  S. aureus-derived orfX and SCCmec included in M. smegmatis
atgaaaatcaccattttagctgtagggaaactaaaagagaaatattggaagcaagccatagcagaatatgaaaaacgtttaggcccatacaccaagatagacatcatagaagttacagacgaaaaagcaccagaaaatatgagcgacaaagaaatcgagcaagtaaaagaaaaagaaggccaacgaatactagccaaaatcaaaccacaatccacagtcattacattagaaatacaaggaaagatgctatcttccgaaggattggcccaagaattgaaccaacgcatgacccaagggcaaagcgactttgtattcgtcattggcggatcaaacggcctgcacaaggacgtcttacaacgtagtaactacgcactatcattcagcaaaatgacatttccacatcaaatgatgcgggttgtgttaattgaacaagtgtacagagcatttaagattatgcgtggagaagcatatcataaatgatgcggttttttcagccgcttcataaagggattttgaatgtatcagaacatatgaggtttatgtgaattgctgttatgtttttaagaagcttatcataagtaatgaggttcatgatttttgacatagttagcctccgcagtctttcatttcaagtaaataatagcgaaatattctttatactgaatacttatagtgaagcaaagttctagctttgagaaaattctttctgcaactaaatatagtaaattacggtaaaatataaataagtacatattgaagaaaatgagacataatatattttataataggagggaatttcaaatgatagacaactttatgcaggtccttaaattaattaaagagaaacgtaccaataatgtagttaaaaaatctgattgggataaaggtgatctatataaaactttagtccatgataagttacccaagcagttaaaagtgcatataaaagaagataaatatga

SEQ ID NO: 9 - DNA, 562 bp, Mycobacterium tuberculosis
gctgaccgaagaagacgtcgtggccaccatcgaatatctggtccgcttgcacgagggtcagaccacgatgaccgttccgggcggcgtcgaggtgccggtggaaaccgacgacatcgaccacttcggcaaccgccgcctgcgtacggtcggcgagctgatccaaaaccagatccgggtcggcatgtcgcggatggagcgggtggtccgggagcggatgaccacccaggacgtggaggcgatcacaccgcagacgttgatcaacatccggccggtggtcgccgcgatcaaggagttcttcggcaccagccagctgagccaattcatggaccagaacaacccgctgtcggggttgacccacaagcgccgactgtcggcgctggggcccggcggtctgtcacgtgagcgtgccgggctggaggtccgcgacgtgcacccgtcgcactacggccggatgtgcccgatcgaaacccctgaggggcccaacatcggtctgatcggctcgctgtcggtgtacgcgcgggtcaacccgttcgggttcatcgaaacgccgtaccgcaaggtg

SEQ ID NO: 10 - DNA, 562 bp, Mycobacterium tuberculosis
gctgaccgaagaagacgtcgtggccaccatcgaatatctggtccgcttgcacgagggtcagaccacgatgaccgttccgggcggcgtcgaggtgccggtggaaaccgacgacatcgaccacttcggcaaccgccgcctgcgtacggtcggcgagctgatccaaaaccagatccgggtcggcatgtcgcggatggagcgggtggtccgggagcggatgaccacccaggacgtggaggcgatcacaccgcagacgttgatcaacatccggccggtggtcgccgcgatcaaggagttcttcggcaccagccagctgagcctattcatggaccagaacaacccgctgtcggggttgacccacaagcgccgactgtcggcgctggggcccggcggtctgtcacgtgagcgtgccgggctggaggtccgcgacgtgcacccgtcgcactacggccggatgtgcccgatcgaaacccctgaggggcccaacatcggtctgatcggctcgctgtcggtgtacgcgcgggtcaacccgttcgggttcatcgaaacgccgtaccgcaaggtg

SEQ ID NO: 11 - DNA, 562 bp, Mycobacterium tuberculosis
gctgaccgaagaagacgtcgtggccaccatcgaatatctggtccgcttgcacgagggtcagaccacgatgaccgttccgggcggcgtcgaggtgccggtggaaaccgacgacatcgaccacttcggcaaccgccgcctgcgtacggtcggcgagctgatccaaaaccagatccgggtcggcatgtcgcggatggagcgggtggtccgggagcggatgaccacccaggacgtggaggcgatcacaccgcagacgttgatcaacatccggccggtggtcgccgcgatcaaggagttcttcggcaccagccagctgagccaattcatggtccagaacaacccgctgtcggggttgacccacaagcgccgactgtcggcgctggggcccggcggtctgtcacgtgagcgtgccgggctggaggtccgcgacgtgcacccgtcgcactacggccggatgtgcccgatcgaaacccctgaggggcccaacatcggtctgatcggctcgctgtcggtgtacgcgcgggtcaacccgttcgggttcatcgaaacgccgtaccgcaaggtg

SEQ ID NO: 12 - DNA, 562 bp, Mycobacterium tuberculosis
gctgaccgaagaagacgtcgtggccaccatcgaatatctggtccgcttgcacgagggtcagaccacgatgaccgttccgggcggcgtcgaggtgccggtggaaaccgacgacatcgaccacttcggcaaccgccgcctgcgtacggtcggcgagctgatccaaaaccagatccgggtcggcatgtcgcggatggagcgggtggtccgggagcggatgaccacccaggacgtggaggcgatcacaccgcagacgttgatcaacatccggccggtggtcgccgcgatcaaggagttcttcggcaccagccagctgagccaattcatggaccagaacaacccgctgtcggggttgacctacaagcgccgactgtcggcgctggggcccggcggtctgtcacgtgagcgtgccgggctggaggtccgcgacgtgcacccgtcgcactacggccggatgtgcccgatcgaaacccctgaggggcccaacatcggtctgatcggctcgctgtcggtgtacgcgcgggtcaacccgttcgggttcatcgaaacgccgtaccgcaaggtg

SEQ ID NO: 13 - DNA, 562 bp, Mycobacterium tuberculosis
gctgaccgaagaagacgtcgtggccaccatcgaatatctggtccgcttgcacgagggtcagaccacgatgaccgttccgggcggcgtcgaggtgccggtggaaaccgacgacatcgaccacttcggcaaccgccgcctgcgtacggtcggcgagctgatccaaaaccagatccgggtcggcatgtcgcggatggagcgggtggtccgggagcggatgaccacccaggacgtggaggcgatcacaccgcagacgttgatcaacatccggccggtggtcgccgcgatcaaggagttcttcggcaccagccagctgagccaattcatggaccagaacaacccgctgtcggggttgacccacaagcgccgactgttggcgctggggcccggcggtctgtcacgtgagcgtgccgggctggaggtccgcgacgtgcacccgtcgcactacggccggatgtgcccgatcgaaacccctgaggggcccaacatcggtctgatcggctcgctgtcggtgtacgcgcgggtcaacccgttcgggttcatcgaaacgccgtaccgcaaggtg

SEQ ID NO: 14 - DNA, 562 bp, Mycobacterium tuberculosis
gctgaccgaagaagacgtcgtggccaccatcgaatatctggtccgcttgcacgagggtcagaccacgatgaccgttccgggcggcgtcgaggtgccggtggaaaccgacgacatcgaccacttcggcaaccgccgcctgcgtacggtcggcgagctgatccaaaaccagatccgggtcggcatgtcgcggatggagcgggtggtccgggagcggatgaccacccaggacgtggaggcgatcacaccgcagacgttgatcaacatccggccggtggtcgccgcgatcaaggagttcttcggcaccagccagctgagccaattcatggaccagaacaacccgctgtcggggttgacccacaagcgccgactgtcggcgccggggcccggcggtctgtcacgtgagcgtgccgggctggaggtccgcgacgtgcacccgtcgcactacggccggatgtgcccgatcgaaacccctgaggggcccaacatcggtctgatcggctcgctgtcggtgtacgcgcgggtcaacccgttcgggttcatcgaaacgccgtaccgcaaggtg